European Patent Specification EP 3 909 972 B1, published February 14, 2024. Title: PD-1-CD28 fusion proteins and their use in medicine. Applicant: Kobold, Sebastian Endres, Stefan. The sequence listing filed with the application follows.

SEQUENCE LISTING (65 sequences)

SEQ ID NO: 1 - DNA, 864 bp, Artificial Sequence
  source 1..864: /mol_type="unassigned DNA" /note="murine full-length PD-1" /organism="Artificial Sequence"
  CDS 1..864: /transl_table=1
atgtgggtgcgccaggtgccgtggagctttacctgggcggtgctgcagctgagctggcagagcggctggctgctggaagtgccgaacggcccgtggcgcagcctgaccttttatccggcgtggctgaccgtgagcgaaggcgcgaacgcgacctttacctgcagcctgagcaactggagcgaagatctgatgctgaactggaaccgcctgagcccgagcaaccagaccgaaaaacaggcggcgttttgcaacggcctgagccagccggtgcaggatgcgcgctttcagattattcagctgccgaaccgccatgattttcatatgaacattctggatacccgccgcaacgatagcggcatttatctgtgcggcgcgattagcctgcatccgaaagcgaaaattgaagaaagcccgggcgcggaactggtggtgaccgaacgcattctggaaaccagcacccgctatccgagcccgagcccgaaaccggaaggccgctttcagggcatggtgattggcattatgagcgcgctggtgggcattccggtgctgctgctgctggcgtgggcgctggcggtgttttgcagcaccagcatgagcgaagcgcgcggcgcgggcagcaaagatgataccctgaaagaagaaccgagcgcggcgccggtgccgagcgtggcgtatgaagaactggattttcagggccgcgaaaaaaccccggaactgccgaccgcgtgcgtgcataccgaatatgcgaccattgtgtttaccgaaggcctgggcgcgagcgcgatgggccgccgcggcagcgcggatggcctgcagggcccgcgcccgccgcgccatgaagatggccattgcagctggccgctg

SEQ ID NO: 2 - protein, 288 aa, Artificial Sequence
  [CDS]:1..864 from SEQ ID NO 1
MWVRQVPWSFTWAVLQLSWQSGWLLEVPNGPWRSLTFYPAWLTVSEGANATFTCSLSNWSEDLMLNWNRLSPSNQTEKQAAFCNGLSQPVQDARFQIIQLPNRHDFHMNILDTRRNDSGIYLCGAISLHPKAKIEESPGAELVVTERILETSTRYPSPSPKPEGRFQGMVIGIMSALVGIPVLLLLAWALAVFCSTSMSEARGAGSKDDTLKEEPSAAPVPSVAYEELDFQGREKTPELPTACVHTEYATIVFTEGLGASAMGRRGSADGLQGPRPPRHEDGHCSWPL

SEQ ID NO: 3 - DNA, 864 bp, Artificial Sequence
  source 1..864: /mol_type="unassigned DNA" /note="human full-length PD-1" /organism="Artificial Sequence"
  CDS 1..864: /transl_table=1
atgcagattccgcaggcgccgtggccggtggtgtgggcggtgctgcagctgggctggcgcccgggctggtttctggatagcccggatcgcccgtggaacccgccgacctttagcccggcgctgctggtggtgaccgaaggcgataacgcgacctttacctgcagctttagcaacaccagcgaaagctttgtgctgaactggtatcgcatgagcccgagcaaccagaccgataaactggcggcgtttccggaagatcgcagccagccgggccaggattgccgctttcgcgtgacccagctgccgaacggccgcgattttcatatgagcgtggtgcgcgcgcgccgcaacgatagcggcacctatctgtgcggcgcgattagcctggcgccgaaagcgcagattaaagaaagcctgcgcgcggaactgcgcgtgaccgaacgccgcgcggaagtgccgaccgcgcatccgagcccgagcccgcgcccggcgggccagtttcagaccctggtggtgggcgtggtgggcggcctgctgggcagcctggtgctgctggtgtgggtgctggcggtgatttgcagccgcgcggcgcgcggcaccattggcgcgcgccgcaccggccagccgctgaaagaagatccgagcgcggtgccggtgtttagcgtggattatggcgaactggattttcagtggcgcgaaaaaaccccggaaccgccggtgccgtgcgtgccggaacagaccgaatatgcgaccattgtgtttccgagcggcatgggcaccagcagcccggcgcgccgcggcagcgcggatggcccgcgcagcgcgcagccgctgcgcccggaagatggccattgcagctggccgctg

SEQ ID NO: 4 - protein, 288 aa, Artificial Sequence
  [CDS]:1..864 from SEQ ID NO 3
MQIPQAPWPVVWAVLQLGWRPGWFLDSPDRPWNPPTFSPALLVVTEGDNATFTCSFSNTSESFVLNWYRMSPSNQTDKLAAFPEDRSQPGQDCRFRVTQLPNGRDFHMSVVRARRNDSGTYLCGAISLAPKAQIKESLRAELRVTERRAEVPTAHPSPSPRPAGQFQTLVVGVVGGLLGSLVLLVWVLAVICSRAARGTIGARRTGQPLKEDPSAVPVFSVDYGELDFQWREKTPEPPVPCVPEQTEYATIVFPSGMGTSSPARRGSADGPRSAQPLRPEDGHCSWPL

SEQ ID NO: 5 - DNA, 570 bp, Artificial Sequence
  source 1..570: /mol_type="unassigned DNA" /note="murine P1 extracellular and transmembrane domain (AA1-190) (PTM construct)" /organism="Artificial Sequence"
  CDS 1..570: /transl_table=1
atgtgggtgcgccaggtgccgtggagctttacctgggcggtgctgcagctgagctggcagagcggctggctgctggaagtgccgaacggcccgtggcgcagcctgaccttttatccggcgtggctgaccgtgagcgaaggcgcgaacgcgacctttacctgcagcctgagcaactggagcgaagatctgatgctgaactggaaccgcctgagcccgagcaaccagaccgaaaaacaggcggcgttttgcaacggcctgagccagccggtgcaggatgcgcgctttcagattattcagctgccgaaccgccatgattttcatatgaacattctggatacccgccgcaacgatagcggcatttatctgtgcggcgcgattagcctgcatccgaaagcgaaaattgaagaaagcccgggcgcggaactggtggtgaccgaacgcattctggaaaccagcacccgctatccgagcccgagcccgaaaccggaaggccgctttcagggcatggtgattggcattatgagcgcgctggtgggcattccggtgctgctgctgctggcgtgggcgctg

SEQ ID NO: 6 - protein, 190 aa, Artificial Sequence
  [CDS]:1..570 from SEQ ID NO 5
MWVRQVPWSFTWAVLQLSWQSGWLLEVPNGPWRSLTFYPAWLTVSEGANATFTCSLSNWSEDLMLNWNRLSPSNQTEKQAAFCNGLSQPVQDARFQIIQLPNRHDFHMNILDTRRNDSGIYLCGAISLHPKAKIEESPGAELVVTERILETSTRYPSPSPKPEGRFQGMVIGIMSALVGIPVLLLLAWAL

SEQ ID NO: 7 - DNA, 507 bp, Artificial Sequence
  source 1..507: /mol_type="unassigned DNA" /note="murine PTM PD-1 extracellular domain (without transmembrane PD-1 domain)" /organism="Artificial Sequence"
  CDS 1..507: /transl_table=1
atgtgggtgcgccaggtgccgtggagctttacctgggcggtgctgcagctgagctggcagagcggctggctgctggaagtgccgaacggcccgtggcgcagcctgaccttttatccggcgtggctgaccgtgagcgaaggcgcgaacgcgacctttacctgcagcctgagcaactggagcgaagatctgatgctgaactggaaccgcctgagcccgagcaaccagaccgaaaaacaggcggcgttttgcaacggcctgagccagccggtgcaggatgcgcgctttcagattattcagctgccgaaccgccatgattttcatatgaacattctggatacccgccgcaacgatagcggcatttatctgtgcggcgcgattagcctgcatccgaaagcgaaaattgaagaaagcccgggcgcggaactggtggtgaccgaacgcattctggaaaccagcacccgctatccgagcccgagcccgaaaccggaaggccgctttcagggcatg

SEQ ID NO: 8 - protein, 169 aa, Artificial Sequence
  [CDS]:1..507 from SEQ ID NO 7
MWVRQVPWSFTWAVLQLSWQSGWLLEVPNGPWRSLTFYPAWLTVSEGANATFTCSLSNWSEDLMLNWNRLSPSNQTEKQAAFCNGLSQPVQDARFQIIQLPNRHDFHMNILDTRRNDSGIYLCGAISLHPKAKIEESPGAELVVTERILETSTRYPSPSPKPEGRFQGM

SEQ ID NO: 9 - DNA, 63 bp, Artificial Sequence
  source 1..63: /mol_type="unassigned DNA" /note="murine PTM PD-1 transmembrane domain" /organism="Artificial Sequence"
  CDS 1..63: /transl_table=1
gtgattggcattatgagcgcgctggtgggcattccggtgctgctgctgctggcgtgggcgctg

SEQ ID NO: 10 - protein, 21 aa, Artificial Sequence
  [CDS]:1..63 from SEQ ID NO 9
VIGIMSALVGIPVLLLLAWAL

SEQ ID NO: 11 - DNA, 123 bp, Artificial Sequence
  source 1..123: /mol_type="unassigned DNA" /note="murine CD28 intracellular domain (AA178-218) (PTM construct)" /organism="Artificial Sequence"
  CDS 1..123: /transl_table=1
aacagccgccgcaaccgcctgctgcagagcgattatatgaacatgaccccgcgccgcccgggcctgacccgcaaaccgtatcagccgtatgcgccggcgcgcgattttgcggcgtatcgcccg

SEQ ID NO: 12 - protein, 41 aa, Artificial Sequence
  [CDS]:1..123 from SEQ ID NO 11
NSRRNRLLQSDYMNMTPRRPGLTRKPYQPYAPARDFAAYRP

SEQ ID NO: 13 - DNA, 693 bp, Artificial Sequence
  source 1..693: /mol_type="unassigned DNA" /note="murine PD1-CD28 (PTM construct)" /organism="Artificial Sequence"
  CDS 1..693: /transl_table=1
atgtgggtgcgccaggtgccgtggagctttacctgggcggtgctgcagctgagctggcagagcggctggctgctggaagtgccgaacggcccgtggcgcagcctgaccttttatccggcgtggctgaccgtgagcgaaggcgcgaacgcgacctttacctgcagcctgagcaactggagcgaagatctgatgctgaactggaaccgcctgagcccgagcaaccagaccgaaaaacaggcggcgttttgcaacggcctgagccagccggtgcaggatgcgcgctttcagattattcagctgccgaaccgccatgattttcatatgaacattctggatacccgccgcaacgatagcggcatttatctgtgcggcgcgattagcctgcatccgaaagcgaaaattgaagaaagcccgggcgcggaactggtggtgaccgaacgcattctggaaaccagcacccgctatccgagcccgagcccgaaaccggaaggccgctttcagggcatggtgattggcattatgagcgcgctggtgggcattccggtgctgctgctgctggcgtgggcgctgaacagccgccgcaaccgcctgctgcagagcgattatatgaacatgaccccgcgccgcccgggcctgacccgcaaaccgtatcagccgtatgcgccggcgcgcgattttgcggcgtatcgcccg

SEQ ID NO: 14 - protein, 231 aa, Artificial Sequence
  [CDS]:1..693 from SEQ ID NO 13
MWVRQVPWSFTWAVLQLSWQSGWLLEVPNGPWRSLTFYPAWLTVSEGANATFTCSLSNWSEDLMLNWNRLSPSNQTEKQAAFCNGLSQPVQDARFQIIQLPNRHDFHMNILDTRRNDSGIYLCGAISLHPKAKIEESPGAELVVTERILETSTRYPSPSPKPEGRFQGMVIGIMSALVGIPVLLLLAWALNSRRNRLLQSDYMNMTPRRPGLTRKPYQPYAPARDFAAYRP

SEQ ID NO: 15 - DNA, 573 bp, Artificial Sequence
  source 1..573: /mol_type="unassigned DNA" /note="human PTM PD-1 extracellular domain plus transmembrane PD-1 domain" /organism="Artificial Sequence"
  CDS 1..573: /transl_table=1
atgcagattccgcaggcgccgtggccggtggtgtgggcggtgctgcagctgggctggcgcccgggctggtttctggatagcccggatcgcccgtggaacccgccgacctttagcccggcgctgctggtggtgaccgaaggcgataacgcgacctttacctgcagctttagcaacaccagcgaaagctttgtgctgaactggtatcgcatgagcccgagcaaccagaccgataaactggcggcgtttccggaagatcgcagccagccgggccaggattgccgctttcgcgtgacccagctgccgaacggccgcgattttcatatgagcgtggtgcgcgcgcgccgcaacgatagcggcacctatctgtgcggcgcgattagcctggcgccgaaagcgcagattaaagaaagcctgcgcgcggaactgcgcgtgaccgaacgccgcgcggaagtgccgaccgcgcatccgagcccgagcccgcgcccggcgggccagtttcagaccctggtggtgggcgtggtgggcggcctgctgggcagcctggtgctgctggtgtgggtgctggcggtgatt

SEQ ID NO: 16 - protein, 191 aa, Artificial Sequence
  [CDS]:1..573 from SEQ ID NO 15
MQIPQAPWPVVWAVLQLGWRPGWFLDSPDRPWNPPTFSPALLVVTEGDNATFTCSFSNTSESFVLNWYRMSPSNQTDKLAAFPEDRSQPGQDCRFRVTQLPNGRDFHMSVVRARRNDSGTYLCGAISLAPKAQIKESLRAELRVTERRAEVPTAHPSPSPRPAGQFQTLVVGVVGGLLGSLVLLVWVLAVI

SEQ ID NO: 17 - DNA, 510 bp, Artificial Sequence
  source 1..510: /mol_type="unassigned DNA" /note="human PD1 extracellular domain (without transmembrane domain) (PD1-CD28 construct)" /organism="Artificial Sequence"
  CDS 1..510: /transl_table=1
atgcagatcccacaggcgccctggccagtcgtctgggcggtgctacaactgggctggcggccaggatggttcttagactccccagacaggccctggaacccccccaccttctccccagccctgctcgtggtgaccgaaggggacaacgccaccttcacctgcagcttctccaacacatcggagagcttcgtgctaaactggtaccgcatgagccccagcaaccagacggacaagctggccgccttccccgaggaccgcagccagcccggccaggactgccgcttccgtgtcacacaactgcccaacgggcgtgacttccacatgagcgtggtcagggcccggcgcaatgacagcggcacctacctctgtggggccatctccctggcccccaaggcgcagatcaaagagagcctgcgggcagagctcagggtgacagagagaagggcagaagtgcccacagcccaccccagcccctcacccaggccagccggccagttccaaaccctggtg

SEQ ID NO: 18 - protein, 170 aa, Artificial Sequence
  [CDS]:1..510 from SEQ ID NO 17
MQIPQAPWPVVWAVLQLGWRPGWFLDSPDRPWNPPTFSPALLVVTEGDNATFTCSFSNTSESFVLNWYRMSPSNQTDKLAAFPEDRSQPGQDCRFRVTQLPNGRDFHMSVVRARRNDSGTYLCGAISLAPKAQIKESLRAELRVTERRAEVPTAHPSPSPRPAGQFQTLV

SEQ ID NO: 19 - DNA, 63 bp, Artificial Sequence
  source 1..63: /mol_type="unassigned DNA" /note="human PD1, transmembrane region (PD1-CD28 construct)" /organism="Artificial Sequence"
  CDS 1..63: /transl_table=1
gttggtgtcgtgggcggcctgctgggcagcctggtgctgctagtctgggtcctggccgtcatc

SEQ ID NO: 20 - protein, 21 aa, Artificial Sequence
  [CDS]:1..63 from SEQ ID NO 19
VGVVGGLLGSLVLLVWVLAVI

SEQ ID NO: 21 - DNA, 126 bp, Artificial Sequence
  source 1..126: /mol_type="unassigned DNA" /note="human CD28 (PD1-CD28 construct)" /organism="Artificial Sequence"
  CDS 1..126: /transl_table=1
aggagtaagaggagcaggctcctgcacagtgactacatgaacatgactccccgccgccccgggcccacccgcaagcattaccagccctatgccccaccacgcgacttcgcagcctatcgctcctaa

SEQ ID NO: 22 - protein, 41 aa, Artificial Sequence
  [CDS]:1..126 from SEQ ID NO 21
RSKRSRLLHSDYMNMTPRRPGPTRKHYQPYAPPRDFAAYRS

SEQ ID NO: 23 - DNA, 699 bp, Artificial Sequence
  source 1..699: /mol_type="unassigned DNA" /note="human PD1-CD28 construct" /organism="Artificial Sequence"
  CDS 1..699: /transl_table=1
atgcagatcccacaggcgccctggccagtcgtctgggcggtgctacaactgggctggcggccaggatggttcttagactccccagacaggccctggaacccccccaccttctccccagccctgctcgtggtgaccgaaggggacaacgccaccttcacctgcagcttctccaacacatcggagagcttcgtgctaaactggtaccgcatgagccccagcaaccagacggacaagctggccgccttccccgaggaccgcagccagcccggccaggactgccgcttccgtgtcacacaactgcccaacgggcgtgacttccacatgagcgtggtcagggcccggcgcaatgacagcggcacctacctctgtggggccatctccctggcccccaaggcgcagatcaaagagagcctgcgggcagagctcagggtgacagagagaagggcagaagtgcccacagcccaccccagcccctcacccaggccagccggccagttccaaaccctggtggttggtgtcgtgggcggcctgctgggcagcctggtgctgctagtctgggtcctggccgtcatcaggagtaagaggagcaggctcctgcacagtgactacatgaacatgactccccgccgccccgggcccacccgcaagcattaccagccctatgccccaccacgcgacttcgcagcctatcgctcctaa

SEQ ID NO: 24 - protein, 232 aa, Artificial Sequence
  [CDS]:1..699 from SEQ ID NO 23
MQIPQAPWPVVWAVLQLGWRPGWFLDSPDRPWNPPTFSPALLVVTEGDNATFTCSFSNTSESFVLNWYRMSPSNQTDKLAAFPEDRSQPGQDCRFRVTQLPNGRDFHMSVVRARRNDSGTYLCGAISLAPKAQIKESLRAELRVTERRAEVPTAHPSPSPRPAGQFQTLVVGVVGGLLGSLVLLVWVLAVIRSKRSRLLHSDYMNMTPRRPGPTRKHYQPYAPPRDFAAYRS

SEQ ID NO: 25 - DNA, 654 bp, Artificial Sequence
  source 1..654: /mol_type="unassigned DNA" /note="murine full-length CD28" /organism="Artificial Sequence"
  CDS 1..654: /transl_table=1
atgaccctgcgcctgctgtttctggcgctgaacttttttagcgtgcaggtgaccgaaaacaaaattctggtgaaacagagcccgctgctggtggtggatagcaacgaagtgagcctgagctgccgctatagctataacctgctggcgaaagaatttcgcgcgagcctgtataaaggcgtgaacagcgatgtggaagtgtgcgtgggcaacggcaactttacctatcagccgcagtttcgcagcaacgcggaatttaactgcgatggcgattttgataacgaaaccgtgacctttcgcctgtggaacctgcatgtgaaccataccgatatttatttttgcaaaattgaatttatgtatccgccgccgtatctggataacgaacgcagcaacggcaccattattcatattaaagaaaaacatctgtgccatacccagagcagcccgaaactgttttgggcgctggtggtggtggcgggcgtgctgttttgctatggcctgctggtgaccgtggcgctgtgcgtgatttggaccaacagccgccgcaaccgcctgctgcagagcgattatatgaacatgaccccgcgccgcccgggcctgacccgcaaaccgtatcagccgtatgcgccggcgcgcgattttgcggcgtatcgcccg

SEQ ID NO: 26 - protein, 218 aa, Artificial Sequence
  [CDS]:1..654 from SEQ ID NO 25
MTLRLLFLALNFFSVQVTENKILVKQSPLLVVDSNEVSLSCRYSYNLLAKEFRASLYKGVNSDVEVCVGNGNFTYQPQFRSNAEFNCDGDFDNETVTFRLWNLHVNHTDIYFCKIEFMYPPPYLDNERSNGTIIHIKEKHLCHTQSSPKLFWALVVVAGVLFCYGLLVTVALCVIWTNSRRNRLLQSDYMNMTPRRPGLTRKPYQPYAPARDFAAYRP

SEQ ID NO: 27 - DNA, 660 bp, Artificial Sequence
  source 1..660: /mol_type="unassigned DNA" /note="human full-length CD28" /organism="Artificial Sequence"
  CDS 1..660: /transl_table=1
atgctgcgcctgctgctggcgctgaacctgtttccgagcattcaggtgaccggcaacaaaattctggtgaaacagagcccgatgctggtggcgtatgataacgcggtgaacctgagctgcaaatatagctataacctgtttagccgcgaatttcgcgcgagcctgcataaaggcctggatagcgcggtggaagtgtgcgtggtgtatggcaactatagccagcagctgcaggtgtatagcaaaaccggctttaactgcgatggcaaactgggcaacgaaagcgtgaccttttatctgcagaacctgtatgtgaaccagaccgatatttatttttgcaaaattgaagtgatgtatccgccgccgtatctggataacgaaaaaagcaacggcaccattattcatgtgaaaggcaaacatctgtgcccgagcccgctgtttccgggcccgagcaaaccgttttgggtgctggtggtggtgggcggcgtgctggcgtgctatagcctgctggtgaccgtggcgtttattattttttgggtgcgcagcaaacgcagccgcctgctgcatagcgattatatgaacatgaccccgcgccgcccgggcccgacccgcaaacattatcagccgtatgcgccgccgcgcgattttgcggcgtatcgcagc

SEQ ID NO: 28 - protein, 220 aa, Artificial Sequence
  [CDS]:1..660 from SEQ ID NO 27
MLRLLLALNLFPSIQVTGNKILVKQSPMLVAYDNAVNLSCKYSYNLFSREFRASLHKGLDSAVEVCVVYGNYSQQLQVYSKTGFNCDGKLGNESVTFYLQNLYVNQTDIYFCKIEVMYPPPYLDNEKSNGTIIHVKGKHLCPSPLFPGPSKPFWVLVVVGGVLACYSLLVTVAFIIFWVRSKRSRLLHSDYMNMTPRRPGPTRKHYQPYAPPRDFAAYRS

SEQ ID NO: 29 - protein, 4 aa, Artificial Sequence
  CD28 domain (not mutated)
YMNM

SEQ ID NO: 30 - protein, 4 aa, Artificial Sequence
  CD28 domain (not mutated)
PYAP

SEQ ID NO: 31 - protein, 4 aa, Artificial Sequence
  CD28 domain (mutated)
FMNM

SEQ ID NO: 32 - protein, 4 aa, Artificial Sequence
  CD28 domain (mutated)
AYAA

SEQ ID NO: 33 - DNA, 870 bp, Artificial Sequence
  source 1..870: /mol_type="unassigned DNA" /note="human PDL-1" /organism="Artificial Sequence"
  CDS 1..870: /transl_table=1
atgcgcatttttgcggtgtttatttttatgacctattggcatctgctgaacgcgtttaccgtgaccgtgccgaaagatctgtatgtggtggaatatggcagcaacatgaccattgaatgcaaatttccggtggaaaaacagctggatctggcggcgctgattgtgtattgggaaatggaagataaaaacattattcagtttgtgcatggcgaagaagatctgaaagtgcagcatagcagctatcgccagcgcgcgcgcctgctgaaagatcagctgagcctgggcaacgcggcgctgcagattaccgatgtgaaactgcaggatgcgggcgtgtatcgctgcatgattagctatggcggcgcggattataaacgcattaccgtgaaagtgaacgcgccgtataacaaaattaaccagcgcattctggtggtggatccggtgaccagcgaacatgaactgacctgccaggcggaaggctatccgaaagcggaagtgatttggaccagcagcgatcatcaggtgctgagcggcaaaaccaccaccaccaacagcaaacgcgaagaaaaactgtttaacgtgaccagcaccctgcgcattaacaccaccaccaacgaaattttttattgcacctttcgccgcctggatccggaagaaaaccataccgcggaactggtgattccggaactgccgctggcgcatccgccgaacgaacgcacccatctggtgattctgggcgcgattctgctgtgcctgggcgtggcgctgacctttatttttcgcctgcgcaaaggccgcatgatggatgtgaaaaaatgcggcattcaggataccaacagcaaaaaacagagcgatacccatctggaagaaacc

SEQ ID NO: 34 - protein, 290 aa, Artificial Sequence
  [CDS]:1..870 from SEQ ID NO 33
MRIFAVFIFMTYWHLLNAFTVTVPKDLYVVEYGSNMTIECKFPVEKQLDLAALIVYWEMEDKNIIQFVHGEEDLKVQHSSYRQRARLLKDQLSLGNAALQITDVKLQDAGVYRCMISYGGADYKRITVKVNAPYNKINQRILVVDPVTSEHELTCQAEGYPKAEVIWTSSDHQVLSGKTTTTNSKREEKLFNVTSTLRINTTTNEIFYCTFRRLDPEENHTAELVIPELPLAHPPNERTHLVILGAILLCLGVALTFIFRLRKGRMMDVKKCGIQDTNSKKQSDTHLEET

SEQ ID NO: 35 - DNA, 819 bp, Artificial Sequence
  source 1..819: /mol_type="unassigned DNA" /note="human PDL-2" /organism="Artificial Sequence"
  CDS 1..819: /transl_table=1
atgatttttctgctgctgatgctgagcctggaactgcagctgcatcagattgcggcgctgtttaccgtgaccgtgccgaaagaactgtatattattgaacatggcagcaacgtgaccctggaatgcaactttgataccggcagccatgtgaacctgggcgcgattaccgcgagcctgcagaaagtggaaaacgataccagcccgcatcgcgaacgcgcgaccctgctggaagaacagctgccgctgggcaaagcgagctttcatattccgcaggtgcaggtgcgcgatgaaggccagtatcagtgcattattatttatggcgtggcgtgggattataaatatctgaccctgaaagtgaaagcgagctatcgcaaaattaacacccatattctgaaagtgccggaaaccgatgaagtggaactgacctgccaggcgaccggctatccgctggcggaagtgagctggccgaacgtgagcgtgccggcgaacaccagccatagccgcaccccggaaggcctgtatcaggtgaccagcgtgctgcgcctgaaaccgccgccgggccgcaactttagctgcgtgttttggaacacccatgtgcgcgaactgaccctggcgagcattgatctgcagagccagatggaaccgcgcacccatccgacctggctgctgcatatttttattccgttttgcattattgcgtttatttttattgcgaccgtgattgcgctgcgcaaacagctgtgccagaaactgtatagcagcaaagataccaccaaacgcccggtgaccaccaccaaacgcgaagtgaacagcgcgatt

SEQ ID NO: 36 - protein, 273 aa, Artificial Sequence
  [CDS]:1..819 from SEQ ID NO 35
MIFLLLMLSLELQLHQIAALFTVTVPKELYIIEHGSNVTLECNFDTGSHVNLGAITASLQKVENDTSPHRERATLLEEQLPLGKASFHIPQVQVRDEGQYQCIIIYGVAWDYKYLTLKVKASYRKINTHILKVPETDEVELTCQATGYPLAEVSWPNVSVPANTSHSRTPEGLYQVTSVLRLKPPPGRNFSCVFWNTHVRELTLASIDLQSQMEPRTHPTWLLHIFIPFCIIAFIFIATVIALRKQLCQKLYSSKDTTKRPVTTTKREVNSAI

SEQ ID NO: 37 - DNA, 870 bp, Artificial Sequence
  source 1..870: /mol_type="unassigned DNA" /note="full length murine PD-L1 (recombinant murine)" /organism="Artificial Sequence"
  CDS 1..870: /transl_table=1
atgcgcatttttgcgggcattatttttaccgcgtgctgccatctgctgcgcgcgtttaccattaccgcgccgaaagatctgtatgtggtggaatatggcagcaacgtgaccatggaatgccgctttccggtggaacgcgaactggatctgctggcgctggtggtgtattgggaaaaagaagatgaacaggtgattcagtttgtggcgggcgaagaagatctgaaaccgcagcatagcaactttcgcggccgcgcgagcctgccgaaagatcagctgctgaaaggcaacgcggcgctgcagattaccgatgtgaaactgcaggatgcgggcgtgtattgctgcattattagctatggcggcgcggattataaacgcattaccctgaaagtgaacgcgccgtatcgcaaaattaaccagcgcattagcgtggatccggcgaccagcgaacatgaactgatttgccaggcggaaggctatccggaagcggaagtgatttggaccaacagcgatcatcagccggtgagcggcaaacgcagcgtgaccaccagccgcaccgaaggcatgctgctgaacgtgaccagcagcctgcgcgtgaacgcgaccgcgaacgatgtgttttattgcaccttttggcgcagccagccgggccagaaccataccgcggaactgattattccggaactgccggcgacccatccgccgcagaaccgcacccattgggtgctgctgggcagcattctgctgtttctgattgtggtgagcaccgtgctgctgtttctgcgcaaacaggtgcgcatgctggatgtggaaaaatgcggcgtggaagataccagcagcaaaaaccgcaacgatacccagtttgaagaaacc

SEQ ID NO: 38 - protein, 290 aa, Artificial Sequence
  [CDS]:1..870 from SEQ ID NO 37
MRIFAGIIFTACCHLLRAFTITAPKDLYVVEYGSNVTMECRFPVERELDLLALVVYWEKEDEQVIQFVAGEEDLKPQHSNFRGRASLPKDQLLKGNAALQITDVKLQDAGVYCCIISYGGADYKRITLKVNAPYRKINQRISVDPATSEHELICQAEGYPEAEVIWTNSDHQPVSGKRSVTTSRTEGMLLNVTSSLRVNATANDVFYCTFWRSQPGQNHTAELIIPELPATHPPQNRTHWVLLGSILLFLIVVSTVLLFLRKQVRMLDVEKCGVEDTSSKNRNDTQFEET

SEQ ID NO: 39 - DNA, 507 bp, Artificial Sequence; identical to SEQ ID NO: 7
  source 1..507: /mol_type="unassigned DNA" /note="murine PD-1 (AA1-169) (CTM construct)" /organism="Artificial Sequence"
  CDS 1..507: /transl_table=1

SEQ ID NO: 40 - protein, 169 aa, Artificial Sequence; identical to SEQ ID NO: 8
  [CDS]:1..507 from SEQ ID NO 39

SEQ ID NO: 41 - DNA, 204 bp, Artificial Sequence
  source 1..204: /mol_type="unassigned DNA" /note="murine CD28 (AA151-218) (CTM construct)" /organism="Artificial Sequence"
  CDS 1..204: /transl_table=1
ttttgggcgctggtggtggtggcgggcgtgctgttttgctatggcctgctggtgaccgtggcgctgtgcgtgatttggaccaacagccgccgcaaccgcctgctgcagagcgattatatgaacatgaccccgcgccgcccgggcctgacccgcaaaccgtatcagccgtatgcgccggcgcgcgattttgcggcgtatcgcccg

SEQ ID NO: 42 - protein, 68 aa, Artificial Sequence
  [CDS]:1..204 from SEQ ID NO 41
FWALVVVAGVLFCYGLLVTVALCVIWTNSRRNRLLQSDYMNMTPRRPGLTRKPYQPYAPARDFAAYRP

SEQ ID NO: 43 - DNA, 711 bp, Artificial Sequence
  source 1..711: /mol_type="unassigned DNA" /note="murine PD1-CD28 (CTM construct)" /organism="Artificial Sequence"
  CDS 1..711: /transl_table=1
atgtgggtgcgccaggtgccgtggagctttacctgggcggtgctgcagctgagctggcagagcggctggctgctggaagtgccgaacggcccgtggcgcagcctgaccttttatccggcgtggctgaccgtgagcgaaggcgcgaacgcgacctttacctgcagcctgagcaactggagcgaagatctgatgctgaactggaaccgcctgagcccgagcaaccagaccgaaaaacaggcggcgttttgcaacggcctgagccagccggtgcaggatgcgcgctttcagattattcagctgccgaaccgccatgattttcatatgaacattctggatacccgccgcaacgatagcggcatttatctgtgcggcgcgattagcctgcatccgaaagcgaaaattgaagaaagcccgggcgcggaactggtggtgaccgaacgcattctggaaaccagcacccgctatccgagcccgagcccgaaaccggaaggccgctttcagggcatgttttgggcgctggtggtggtggcgggcgtgctgttttgctatggcctgctggtgaccgtggcgctgtgcgtgatttggaccaacagccgccgcaaccgcctgctgcagagcgattatatgaacatgaccccgcgccgcccgggcctgacccgcaaaccgtatcagccgtatgcgccggcgcgcgattttgcggcgtatcgcccg

SEQ ID NO: 44 - protein, 237 aa, Artificial Sequence
  [CDS]:1..711 from SEQ ID NO 43
MWVRQVPWSFTWAVLQLSWQSGWLLEVPNGPWRSLTFYPAWLTVSEGANATFTCSLSNWSEDLMLNWNRLSPSNQTEKQAAFCNGLSQPVQDARFQIIQLPNRHDFHMNILDTRRNDSGIYLCGAISLHPKAKIEESPGAELVVTERILETSTRYPSPSPKPEGRFQGMFWALVVVAGVLFCYGLLVTVALCVIWTNSRRNRLLQSDYMNMTPRRPGLTRKPYQPYAPARDFAAYRP

SEQ ID NO: 45 - DNA, 507 bp, Artificial Sequence; identical to SEQ ID NO: 7
  source 1..507: /mol_type="unassigned DNA" /note="murine PD1 (AA1-169) (CEX construct)" /organism="Artificial Sequence"
  CDS 1..507: /transl_table=1

SEQ ID NO: 46 - protein, 169 aa, Artificial Sequence; identical to SEQ ID NO: 8
  [CDS]:1..507 from SEQ ID NO 45

SEQ ID NO: 47 - DNA, 312 bp, Artificial Sequence
  source 1..312: /mol_type="unassigned DNA" /note="murine CD28 (AA115-218) (CEX construct)" /organism="Artificial Sequence"
  CDS 1..312: /transl_table=1
attgaatttatgtatccgccgccgtatctggataacgaacgcagcaacggcaccattattcatattaaagaaaaacatctgtgccatacccagagcagcccgaaactgttttgggcgctggtggtggtggcgggcgtgctgttttgctatggcctgctggtgaccgtggcgctgtgcgtgatttggaccaacagccgccgcaaccgcctgctgcagagcgattatatgaacatgaccccgcgccgcccgggcctgacccgcaaaccgtatcagccgtatgcgccggcgcgcgattttgcggcgtatcgcccg

SEQ ID NO: 48 - protein, 104 aa, Artificial Sequence
  [CDS]:1..312 from SEQ ID NO 47
IEFMYPPPYLDNERSNGTIIHIKEKHLCHTQSSPKLFWALVVVAGVLFCYGLLVTVALCVIWTNSRRNRLLQSDYMNMTPRRPGLTRKPYQPYAPARDFAAYRP

SEQ ID NO: 49 - DNA, 819 bp, Artificial Sequence
  source 1..819: /mol_type="unassigned DNA" /note="murine PD1-CD28 (CEX construct)" /organism="Artificial Sequence"
  CDS 1..819: /transl_table=1
atgtgggtgcgccaggtgccgtggagctttacctgggcggtgctgcagctgagctggcagagcggctggctgctggaagtgccgaacggcccgtggcgcagcctgaccttttatccggcgtggctgaccgtgagcgaaggcgcgaacgcgacctttacctgcagcctgagcaactggagcgaagatctgatgctgaactggaaccgcctgagcccgagcaaccagaccgaaaaacaggcggcgttttgcaacggcctgagccagccggtgcaggatgcgcgctttcagattattcagctgccgaaccgccatgattttcatatgaacattctggatacccgccgcaacgatagcggcatttatctgtgcggcgcgattagcctgcatccgaaagcgaaaattgaagaaagcccgggcgcggaactggtggtgaccgaacgcattctggaaaccagcacccgctatccgagcccgagcccgaaaccggaaggccgctttcagggcatgattgaatttatgtatccgccgccgtatctggataacgaacgcagcaacggcaccattattcatattaaagaaaaacatctgtgccatacccagagcagcccgaaactgttttgggcgctggtggtggtggcgggcgtgctgttttgctatggcctgctggtgaccgtggcgctgtgcgtgatttggaccaacagccgccgcaaccgcctgctgcagagcgattatatgaacatgaccccgcgccgcccgggcctgacccgcaaaccgtatcagccgtatgcgccggcgcgcgattttgcggcgtatcgcccg

SEQ ID NO: 50 - protein, 273 aa, Artificial Sequence
  [CDS]:1..819 from SEQ ID NO 49
MWVRQVPWSFTWAVLQLSWQSGWLLEVPNGPWRSLTFYPAWLTVSEGANATFTCSLSNWSEDLMLNWNRLSPSNQTEKQAAFCNGLSQPVQDARFQIIQLPNRHDFHMNILDTRRNDSGIYLCGAISLHPKAKIEESPGAELVVTERILETSTRYPSPSPKPEGRFQGMIEFMYPPPYLDNERSNGTIIHIKEKHLCHTQSSPKLFWALVVVAGVLFCYGLLVTVALCVIWTNSRRNRLLQSDYMNMTPRRPGLTRKPYQPYAPARDFAAYRP

SEQ ID NO: 51 - DNA, 693 bp, Artificial Sequence
  source 1..693: /mol_type="unassigned DNA" /note="PTM-FMNM construct (murine)" /organism="Artificial Sequence"
  CDS 1..693: /transl_table=1
atgtgggtgcgccaggtgccgtggagctttacctgggcggtgctgcagctgagctggcagagcggctggctgctggaagtgccgaacggcccgtggcgcagcctgaccttttatccggcgtggctgaccgtgagcgaaggcgcgaacgcgacctttacctgcagcctgagcaactggagcgaagatctgatgctgaactggaaccgcctgagcccgagcaaccagaccgaaaaacaggcggcgttttgcaacggcctgagccagccggtgcaggatgcgcgctttcagattattcagctgccgaaccgccatgattttcatatgaacattctggatacccgccgcaacgatagcggcatttatctgtgcggcgcgattagcctgcatccgaaagcgaaaattgaagaaagcccgggcgcggaactggtggtgaccgaacgcattctggaaaccagcacccgctatccgagcccgagcccgaaaccggaaggccgctttcagggcatggtgattggcattatgagcgcgctggtgggcattccggtgctgctgctgctggcgtgggcgctgaacagccgccgcaaccgcctgctgcagagcgattttatgaacatgaccccgcgccgcccgggcctgacccgcaaaccgtatcagccgtatgcgccggcgcgcgattttgcggcgtatcgcccg

SEQ ID NO: 52 - protein, 231 aa, Artificial Sequence
  [CDS]:1..693 from SEQ ID NO 51
MWVRQVPWSFTWAVLQLSWQSGWLLEVPNGPWRSLTFYPAWLTVSEGANATFTCSLSNWSEDLMLNWNRLSPSNQTEKQAAFCNGLSQPVQDARFQIIQLPNRHDFHMNILDTRRNDSGIYLCGAISLHPKAKIEESPGAELVVTERILETSTRYPSPSPKPEGRFQGMVIGIMSALVGIPVLLLLAWALNSRRNRLLQSDFMNMTPRRPGLTRKPYQPYAPARDFAAYRP

SEQ ID NO: 53 - DNA, 693 bp, Artificial Sequence
  source 1..693: /mol_type="unassigned DNA" /note="PTM-AYAA construct (murine)" /organism="Artificial Sequence"
  CDS 1..693: /transl_table=1
atgtgggtgcgccaggtgccgtggagctttacctgggcggtgctgcagctgagctggcagagcggctggctgctggaagtgccgaacggcccgtggcgcagcctgaccttttatccggcgtggctgaccgtgagcgaaggcgcgaacgcgacctttacctgcagcctgagcaactggagcgaagatctgatgctgaactggaaccgcctgagcccgagcaaccagaccgaaaaacaggcggcgttttgcaacggcctgagccagccggtgcaggatgcgcgctttcagattattcagctgccgaaccgccatgattttcatatgaacattctggatacccgccgcaacgatagcggcatttatctgtgcggcgcgattagcctgcatccgaaagcgaaaattgaagaaagcccgggcgcggaactggtggtgaccgaacgcattctggaaaccagcacccgctatccgagcccgagcccgaaaccggaaggccgctttcagggcatggtgattggcattatgagcgcgctggtgggcattccggtgctgctgctgctggcgtgggcgctgaacagccgccgcaaccgcctgctgcagagcgattatatgaacatgaccccgcgccgcccgggcctgacccgcaaaccgtatcaggcgtatgcggcggcgcgcgattttgcggcgtatcgcccg

SEQ ID NO: 54 - protein, 231 aa, Artificial Sequence
  [CDS]:1..693 from SEQ ID NO 53
MWVRQVPWSFTWAVLQLSWQSGWLLEVPNGPWRSLTFYPAWLTVSEGANATFTCSLSNWSEDLMLNWNRLSPSNQTEKQAAFCNGLSQPVQDARFQIIQLPNRHDFHMNILDTRRNDSGIYLCGAISLHPKAKIEESPGAELVVTERILETSTRYPSPSPKPEGRFQGMVIGIMSALVGIPVLLLLAWALNSRRNRLLQSDYMNMTPRRPGLTRKPYQAYAAARDFAAYRP

SEQ ID NO: 55 - DNA, 693 bp, Artificial Sequence
  source 1..693: /mol_type="unassigned DNA" /note="PTM-FMNM-AYAA construct (murine)" /organism="Artificial Sequence"
  CDS 1..693: /transl_table=1
atgtgggtgcgccaggtgccgtggagctttacctgggcggtgctgcagctgagctggcagagcggctggctgctggaagtgccgaacggcccgtggcgcagcctgaccttttatccggcgtggctgaccgtgagcgaaggcgcgaacgcgacctttacctgcagcctgagcaactggagcgaagatctgatgctgaactggaaccgcctgagcccgagcaaccagaccgaaaaacaggcggcgttttgcaacggcctgagccagccggtgcaggatgcgcgctttcagattattcagctgccgaaccgccatgattttcatatgaacattctggatacccgccgcaacgatagcggcatttatctgtgcggcgcgattagcctgcatccgaaagcgaaaattgaagaaagcccgggcgcggaactggtggtgaccgaacgcattctggaaaccagcacccgctatccgagcccgagcccgaaaccggaaggccgctttcagggcatggtgattggcattatgagcgcgctggtgggcattccggtgctgctgctgctggcgtgggcgctgaacagccgccgcaaccgcctgctgcagagcgattttatgaacatgaccccgcgccgcccgggcctgacccgcaaaccgtatcaggcgtatgcggcggcgcgcgattttgcggcgtatcgcccg

SEQ ID NO: 56 - protein, 231 aa, Artificial Sequence
  [CDS]:1..693 from SEQ ID NO 55
MWVRQVPWSFTWAVLQLSWQSGWLLEVPNGPWRSLTFYPAWLTVSEGANATFTCSLSNWSEDLMLNWNRLSPSNQTEKQAAFCNGLSQPVQDARFQIIQLPNRHDFHMNILDTRRNDSGIYLCGAISLHPKAKIEESPGAELVVTERILETSTRYPSPSPKPEGRFQGMVIGIMSALVGIPVLLLLAWALNSRRNRLLQSDFMNMTPRRPGLTRKPYQAYAAARDFAAYRP

SEQ ID NO: 57 - DNA, 741 bp, Artificial Sequence
  source 1..741: /mol_type="unassigned DNA" /note="murine PD1 deletion mutant" /organism="Artificial Sequence"
  CDS 1..741: /transl_table=1
atgtgggtgcgccaggtgccgtggagctttacctgggcggtgctgcagctgagctggcagagcggctggctgctggaagtgccgaacggcccgtggcgcagcctgaccttttatccggcgtggctgaccgtgagcgaaggcgcgaacgcgacctttacctgcagcctgagcaactggagcgaagatctgatgctgaactggaaccgcctgagcccgagcaaccagaccgaaaaacaggcggcgttttgcaacggcctgagccagccggtgcaggatgcgcgctttcagattattcagctgccgaaccgccatgattttcatatgaacattctggatacccgccgcaacgatagcggcatttatctgtgcggcgcgattagcctgcatccgaaagcgaaaattgaagaaagcccgggcgcggaactggtggtgaccgaacgcattctggaaaccagcacccgctatccgagcccgagcccgaaaccggaaggccgctttcagggcatggtgattggcattatgagcgcgctggtgggcattccggtgctgctgctgctggcgtgggcgctggcggtgttttgcagcaccagcatgagcgaagcgcgcggcgcgggcagcaaagatgataccctgaaagaagaaccgagcgcggcgccggtgccgagcgtggcgtatgaagaactggattttcagggccgcgaaaaaaccccggaactgccgaccgcgtgcgtgcataccgaa

SEQ ID NO: 58 - protein, 247 aa, Artificial Sequence
  [CDS]:1..741 from SEQ ID NO 57
MWVRQVPWSFTWAVLQLSWQSGWLLEVPNGPWRSLTFYPAWLTVSEGANATFTCSLSNWSEDLMLNWNRLSPSNQTEKQAAFCNGLSQPVQDARFQIIQLPNRHDFHMNILDTRRNDSGIYLCGAISLHPKAKIEESPGAELVVTERILETSTRYPSPSPKPEGRFQGMVIGIMSALVGIPVLLLLAWALAVFCSTSMSEARGAGSKDDTLKEEPSAAPVPSVAYEELDFQGREKTPELPTACVHTE

SEQ ID NO: 59 - DNA, 29 bp, Artificial Sequence
  source 1..29: /mol_type="unassigned DNA" /note="Primer" /organism="Artificial Sequence"
atagcggccgcgccaccatgtgggtccgg

SEQ ID NO: 60 - DNA, 23 bp, Artificial Sequence
  source 1..23: /mol_type="unassigned DNA" /note="Primer" /organism="Artificial Sequence"
ccttctactattgcagaagacag

SEQ ID NO: 61 - DNA, 23 bp, Artificial Sequence
  source 1..23: /mol_type="unassigned DNA" /note="Primer" /organism="Artificial Sequence"
ctgtcttctgcaatagtagaagg

SEQ ID NO: 62 - DNA, 28 bp, Artificial Sequence
  source 1..28: /mol_type="unassigned DNA" /note="Primer" /organism="Artificial Sequence"
tatgaattctcaggggcggtacgctgca

SEQ ID NO: 63 - DNA, 29 bp, Artificial Sequence
  source 1..29: /mol_type="unassigned DNA" /note="Primer" /organism="Artificial Sequence"
atagcggccgcgccaccatgtgggtccgg

SEQ ID NO: 64 - DNA, 28 bp, Artificial Sequence
  source 1..28: /mol_type="unassigned DNA" /note="Primer" /organism="Artificial Sequence"
tatgaattctcaggggcggtacgctgca

SEQ ID NO: 65 - protein, 8 aa, Artificial Sequence
  Control peptide
SIINFEKL